European Patent Application EP 4 647 438 A1, published November 12, 2025. Title: Polypeptide comprising a capsid protein sequence. Applicant: A-Spectar GmbH. Application EP, filed May 8, 2024. The sequence listing filed with the application follows.

SEQUENCE LISTING (5 sequences)

SEQ ID NO: 1 - protein, 644 aa, Nudaurelia capensis omega virus
MDSNSASGKRRSRNVRIAANTVNVAPKQRQARGRRARSRANNIDNVTAAAQELGQSLDANVITFPTNVATMPEFRSWARGKLDIDQDSIGWYFKYLDPAGATESARAVGEYSKIPDGLVKFSVDAEIREIYNEECPTVSDASIPLDGAQWSLSIISYPMFRTAYFAVANVDNKEISLDVTNDLIVWLNNLASWRDVVDSGQWFTFSDDPTWFVRIRVLHPTYDLPDPTEGLLRTCSDYRLTYKSITCEANMPTLVDQGFWIGGHYALTPIATTQNAVEGSGFEHPFNVTRPGIAAGVTLTWASMPPGGSAPSGDPAWIPDSTTQFQWRHGGFDAPTGVITYTIPRGYTMQYFDTTTNEWNGFANPDDVVTFGQTGGAAGTNATITITAPTVTLTILATTTSAANVINFRNLDAETTAASNRSEVPLPPLTFGQTAPNNPKIEQTLVKDTLGSYLVHSKMRNPVFQLTPASSFGAISFTNPGFDRNLDLPGFGGIRDSLDVNMSTAVCHFRSLSKSCSIVTKTYQGWEGVTNVNTPFGQFAHSGLLKNDEILCLADDLATRLTGVYGATDNFAAAVLAFAANMLTSVLKSEATTSVIKELGNQATGLANQGLARLPGLLASIPGKIAARVRARRDRRRAARMNNN

SEQ ID NO: 2 - protein, 647 aa, Helicoverpa armigera stunt virus
MGDAGVASQRPHNRRGTRNVRVSANTVTVNGRRNQRRRTGRQVSPPDNFTAAAQDLAQSLDANTVTFPANISSMPEFRNWAKGKIDLDSDSIGWYFKYLDPAGATESARAVGEYSKIPDGLVKFSVDAEIREIYNEECPVVTDVSVPLDGRQWSLSIFSFPMFRTAYVAVANVENKEMSLDVVNDLIEWLNNLADWRYVVDSEQWINFTNDTTYYVRIRVLRPTYDVPDPTEGLVRTVSDYRLTYKAITCEANMPTLVDQGFWIGGQYALTPTSLPQYDVSEAYALHTLTFARPSSAAALAFVWAGLPQGGTAPAGTPAWEQASSGGYLTWRHNGTTFPAGSVSYVLPEGFALERYDPNDGSWTDFASAGDTVTFRQVAVDEVVVTNNPAGGGSAPTFTVRVPPSNAYTNTVFRNTLLETRPSSRRLELPMPPADFGQTVANNPKIEQSLLKETLGCYLVHSKMRNPVFQLTPASSFGAVSFNNPGYERTRDLPDYTGIRDSFDQNMSTAVAHFRSLSHSCSIVTKTYQGWEGVTNVNTPFGQFAHAGLLKNEEILCLADDLATRLTGVYPATDNFAAAVSAFAANMLSSVLKSEATSSIIKSVGETAVGAAQSGLAKLPGLLMSVPGKIAARVRARRARRRAARAN

SEQ ID NO: 3 - protein, 15 aa, synthetic construct
  REGION 1..15: note = CPP
RRRRNRTRRNRRRVR

SEQ ID NO: 4 - protein, 11 aa, synthetic construct
  REGION 1..11: note = MC11-peptide
MQLPLATGGGC

SEQ ID NO: 5 - protein, 12 aa, synthetic construct
  REGION 1..12: note = GE11-peptide
YHWYGYTPQNVI